European Patent Application EP 4 790 144 A1, published August 12, 2026. Title: 一种新生物标志物在诊断或辅助诊断SPN中的应用. Applicant: 中国医学科学院北京协和医院. Application WO. The sequence listing filed with the application follows.

SEQUENCE LISTING (57 sequences)

SEQ ID NO: 1 - protein, 8 aa, synthetic construct
GYAFTNYG

SEQ ID NO: 2 - protein, 8 aa, synthetic construct
GFTFSDAW

SEQ ID NO: 3 - protein, 8 aa, synthetic construct
GFTFSTYA

SEQ ID NO: 4 - protein, 8 aa, synthetic construct
GYTFTDFG

SEQ ID NO: 5 - protein, 8 aa, synthetic construct
GYTFTDYV

SEQ ID NO: 6 - protein, 8 aa, synthetic construct
GLTFSIYA

SEQ ID NO: 7 - protein, 8 aa, synthetic construct
GYTFTRYY

SEQ ID NO: 8 - protein, 8 aa, synthetic construct
GFTFSIYA

SEQ ID NO: 9 - protein, 8 aa, synthetic construct
IKTYTGDS

SEQ ID NO: 10 - protein, 10 aa, synthetic construct
IRSKAINHAT

SEQ ID NO: 11 - protein, 8 aa, synthetic construct
ISSGGSST

SEQ ID NO: 12 - protein, 8 aa, synthetic construct
INTYTGDP

SEQ ID NO: 13 - protein, 8 aa, synthetic construct
INTYSGET

SEQ ID NO: 14 - protein, 8 aa, synthetic construct
INTYTGAT

SEQ ID NO: 15 - protein, 8 aa, synthetic construct
IYPGSGST

SEQ ID NO: 16 - protein, 8 aa, synthetic construct
ISAGDIYP

SEQ ID NO: 17 - protein, 8 aa, synthetic construct
INPTNGVA

SEQ ID NO: 18 - protein, 12 aa, synthetic construct
VREPIYYGWVDY

SEQ ID NO: 19 - protein, 10 aa, synthetic construct
TRRVDWYFDV

SEQ ID NO: 20 - protein, 12 aa, synthetic construct
ARHGDWDGSLAY

SEQ ID NO: 21 - protein, 12 aa, synthetic construct
VREPLYYGWVDY

SEQ ID NO: 22 - protein, 14 aa, synthetic construct
ARSYDYDGLAWFAY

SEQ ID NO: 23 - protein, 9 aa, synthetic construct
TSITMAMAY

SEQ ID NO: 24 - protein, 12 aa, synthetic construct
TRVYYKYDGFAY

SEQ ID NO: 25 - protein, 11 aa, synthetic construct
KSLLHRNGNTY

SEQ ID NO: 26 - protein, 6 aa, synthetic construct
QSIGTS

SEQ ID NO: 27 - protein, 6 aa, synthetic construct
QDVNAA

SEQ ID NO: 28 - protein, 11 aa, synthetic construct
KSLLHSNGNTY

SEQ ID NO: 29 - protein, 11 aa, synthetic construct
QSLLYSNGKTY

SEQ ID NO: 30 - protein, 6 aa, synthetic construct
QDVGTA

SEQ ID NO: 31 - protein, 9 aa, synthetic construct
MQHLEYPYT

SEQ ID NO: 32 - protein, 9 aa, synthetic construct
QQSNSWPLT

SEQ ID NO: 33 - protein, 9 aa, synthetic construct
QQHYSAPRT

SEQ ID NO: 34 - protein, 9 aa, synthetic construct
WQGAHFPWT

SEQ ID NO: 35 - protein, 9 aa, synthetic construct
QQYSSYPLT

SEQ ID NO: 36 - protein, 119 aa, synthetic construct
QLQLVQSGPEVKKPGETVKISCKASGYAFTNYGMNWVKQAPGKDLKWMGWIKTYTGDSVYGDDFKGRFAFSLDTSASTAYLQINDLKNEDTATYFCVREPIYYGWVDYWGQGTSVTVSS

SEQ ID NO: 37 - protein, 119 aa, synthetic construct
EVKLEESGGGLVQPGGSMKLSCGASGFTFSDAWMDWVRQSPEKGLEWVAEIRSKAINHATYYAESVKGRFTISRDDSKSSVYLQMNSLRAEDTGIYYCTRRVDWYFDVWGAGTTVTVSS

SEQ ID NO: 38 - protein, 119 aa, synthetic construct
IVMLVESGGGLVKPGGSLKLSCVASGFTFSTYAMSWIRQTPEKRLAWVATISSGGSSTYYSDSVKGRFTISRDNAKNTLYLQMSSLRSEDTAMYYCARHGDWDGSLAYWGQGTQVTVSA

SEQ ID NO: 39 - protein, 119 aa, synthetic construct
QLQLVQSGPEVKKPGETVKISCKASGYAFTNYGMNWVKQAPGKDLKWMGWINTYTGDPVYGDDFKGRFAFSLDTSASTAYLQINNLKNEDTATYFCVREPIYYGWVDYWGQGTSVTVSS

SEQ ID NO: 40 - protein, 119 aa, synthetic construct
QLQLVQSGPELKKPGETVKISCKASGYAFTNYGMNWVKQTPGKGLKWMGWINTYSGETTYGDDFKGRFAFSLETSASTAYLQINSLKNEDTATYFCVREPIYYGWVDYWGQGTSVTVSS

SEQ ID NO: 41 - protein, 119 aa, synthetic construct
QIQLVQSGPELKKPGETVKISCKTSGYTFTDFGMNWVKRAPGQDLKWMGWINTYTGATTYGDEFKGRFAFSLETSASTASLQINNLKNEDSATYFCVREPLYYGWVDYWGQGTSVIVSS

SEQ ID NO: 42 - protein, 121 aa, synthetic construct
QVQLQQSGPELVKPGASVKMSCKASGYTFTDYVISWVKQRTGQGLEWIGEIYPGSGSTYYNEKFKGKATLTADKSSNTAYMQLSSLTSEDSAVYFCARSYDYDGLAWFAYWGQGTLVTVSA

SEQ ID NO: 43 - protein, 116 aa, synthetic construct
DVKLVESGGGLVKPGGSLKLSCAASGLTFSIYAMSWVRQTPEKRLEWVATISAGDIYPYYSDSVKGRFAISRDNAKNTLYLQMSSLRSEDTAIYYCTSITMAMAYWGQGTLVTVSA

SEQ ID NO: 44 - protein, 119 aa, synthetic construct
QVQLQQSGAELVKPGASVKLSCKASGYTFTRYYLYWVKQRPGQGLEWIGKINPTNGVADLNEKFKYKATLTVDKSSSTTHMQLSSLTSEDSAVYYCTRVYYKYDGFAYWGQGTLVTVSA

SEQ ID NO: 45 - protein, 116 aa, synthetic construct
DVKLVESGGGLVKPGGSLKLSCAASGFTFSIYAMSWVRQTPEKRLEWVATISAGDIYPYYSDSVKGRFAISRDNAKNTLFLQMSSLRSEDTAIYYCTSITMAMAYWGQGTLVTVSA

SEQ ID NO: 46 - protein, 112 aa, synthetic construct
DIVMTQAAPSVPVTPGESASISCRSSKSLLHRNGNTYLYWFLQRPGQSPQVLIYRMSNLASGVPDRFSGSGSGTAFTLRISRVEAEDVGVYYCMQHLEYPYTFGGGTKLEIK

SEQ ID NO: 47 - protein, 107 aa, synthetic construct
DILLTQSPAILSVSPGERVSFSCRASQSIGTSIYWYQQRTNGSPRLLIKYASESISGIPSRFSGSGSGTDFTLSINSVESEDIADYYCQQSNSWPLTFGAGTKLELK

SEQ ID NO: 48 - protein, 107 aa, synthetic construct
DIVMTQSHKLMSTSVGDRVNITCKASQDVNAAVAWYQQQPGQSPKLLFYWASTRHTGVPDRFTGSGSRTDYTLTISGVQAEDLALYYCQQHYSAPRTFGGGTKLEVK

SEQ ID NO: 49 - protein, 112 aa, synthetic construct; identical to SEQ ID NO: 46

SEQ ID NO: 50 - protein, 112 aa, synthetic construct
DIVMTQAAPSVPVTPGESVSISCRSSKSLLHRNGNTYLYWFLQRPGQSPQVLIYRMSNLASGVPDRFSGSGSGTAFTLRISRVEAEDVGVYYCMQHLEYPYTFGGGTKLEIK

SEQ ID NO: 51 - protein, 112 aa, synthetic construct
DIVMTQVAPSVPVTPGESVSISCRSSKSLLHRNGNTYLYWFLQRPGQSPQVLIYRMSNLASGVPDRFSGSGSGTAFTLRISRVEAEDVGVYYCMQHLEYPYTFGGGTKLEIK

SEQ ID NO: 52 - protein, 112 aa, synthetic construct
DIVMTQAAPSVPVTPGESVSISCRSSKSLLHSNGNTYLYWFLQRPGQSPQLLIYRMSNLASGVPDRFSGSGSGTAFTLRISRVEAEDVGVYYCMQHLEYPLTFGSGTKLEIK

SEQ ID NO: 53 - protein, 112 aa, synthetic construct
DVVMTQTPLTLSVTIGQPASISCKSSQSLLYSNGKTYLSWLLQRPGQSPKRLIYLVSKLDSGVPDRFTGSGSGTEFTLKISRVEAEDLGVYYCWQGAHFPWTFGGGTKLEIK

SEQ ID NO: 54 - protein, 107 aa, synthetic construct
DIVMTQSLKFMSTSVGDRVSIICKASQDVGTAVAWYQQKPAQSPKLLIYWASTRHTGVPDRFTGSGSGTDFTLTISNVQSEDLTDYFCQQYSSYPLTFGGGTKLEIK

SEQ ID NO: 55 - protein, 112 aa, synthetic construct
DVVMTQTPLTLSVTIGQPASISCKSSQSLLYSNGKTYLSWLLQRPGQSPKRLIYLVSKLDSGVPDRFTGSGSGTDFTLKISRVEAEDLGVYYCWQGAHFPWTFGGGTKLEIK

SEQ ID NO: 56 - protein, 96 aa, synthetic construct
AGIALLSITHRPSLWKYHTHLLQFDGEGGWKFEKLDSAARLSLTEEKQRLEQQLAGIPKMQRRLQELCQILGEAVAPAHVPAPSPQGPGGLQGAST

SEQ ID NO: 57 - protein, 19 aa, synthetic construct
CQILGEAVAPAHVPAPSPQ